European Patent Application EP 4 239 074 A1, published September 6, 2023. Title: RECOMBINANT VECTOR AND EXPRESSION AND PURIFICATION METHOD FOR THERMO-LABILE UNG FUSED PROTEIN. Applicant: XIAMEN UNIVERSITY XIAMEN ZEESAN BIOTECH CO., Ltd. The sequence listing filed with the application follows.

SEQUENCE LISTING (5 sequences)

SEQ ID NO: 1 - DNA, 36 bp, Artificial Sequence
  Primer sequence
tagtgagctcggtaccatgttcggagagacttggag

SEQ ID NO: 2 - DNA, 36 bp, Artificial Sequence
  Primer sequence
acctatctagactgcattagagtgctctccagttta

SEQ ID NO: 3 - DNA, 666 bp, Artificial Sequence
  Sequence encoding for the rCod UNG protein
atgttcggagagacttggagaagagagctggctgcagagtttgaaaagccatacttcaaacaattgatgtcctttgtagctgatgagaggagccgtcacaccgtctacccaccggctgatcaagtgtacagttggacagagatgtgtgacattcaagatgtgaaagtagtgattctaggccaggacccttaccacggtcccaaccaagcacatggactctgtttcagtgtgcaaaagccagttccccctccccccagtctcgtgaacatatacaaagaattgtgtaccgacattgatggcttcaagcatcctggacatggagatctaagcggatgggcaaaacaaggggtgctgctgcttaacgcggtgctgaccgtgcgggcccatcaggccaactcccacaaggacagaggctgggagaccttcaccgacgctgtgatcaagtggctgagcgtcaaccgggaaggagtggttttcctgttgtggggctcatacgcccataagaagggagcgaccatcgacaggaaacgtcaccatgtcttgcaagctgttcatccatctcctttgtctgctcatcgtgggttccttggttgtaagcacttctccaaggctaacgggctgctgaaactatctgggacggagcctataaactggagagcactctaa

SEQ ID NO: 4 - DNA, 4740 bp, Artificial Sequence
  Sequence of the pCold-SUMO vector
aaggaatggtgtggccgattaatcataaatatgaaaaataattgttgcatcacccgccaatgcgtggcttaatgcacatcaaattgtgagcggataacaatttgatgtgctagcgcatatccagtgtagtaaggcaagtcccttcaagagttatcgttgatacccctcgtagtgcacattcctttaacgcttcaaaatctgtaaagcacgccatatcgccgaaaggcacacttaattattaagaggtaatacaccatgaatcacaaagtgcatcatcatcatcatcatatcgaaggtaggcatatgggcggtggcggtagcggcggtggcggtagcggtatgtcggactcagaagtcaatcaagaagctaagccagaggtcaagccagaagtcaagcctgagactcacatcaatttaaaggtgtccgatggatcttcagagatcttcttcaagatcaaaaagaccactcctttaagaaggctgatggaagcgttcgctaaaagacagggtaaggaaatggactccttaagattcttgtacgacggtattagaattcaagctgatcagacccctgaagatttggacatggaggataacgatattattgaggctcacagagaacagattggtggtactagtgagctcggtaccctcgagggatccgaattcaagcttgtcgacctgcagtctagataggtaatctctgcttaaaagcacagaatctaagatccctgccatttggcggggatttttttatttgttttcaggaaataaataatcgatcgcgtaataaaatctattattatttttgtgaagaataaatttgggtgcaatgagaatgcgcaggccctttcgtctcgcgcgtttcggtgatgacggtgaaaacctctgacacatgcagctcccggagacggtcacagcttgtctgtaagcggatgccgggagcagacaagcccgtcagggcgcgtcagcgggtgttggcgggtgtcggggctggcttaactatgcggcatcagagcagattgtactgagagtgcaccataaaattgtaaacgttaatattttgttaaaattcgcgttaaatttttgttaaatcagctcattttttaaccaataggccgaaatcggcaaaatcccttataaatcaaaagaatagcccgagatagggttgagtgttgttccagtttggaacaagagtccactattaaagaacgtggactccaacgtcaaagggcgaaaaaccgtctatcagggcgatggcccactacgtgaaccatcacccaaatcaagttttttggggtcgaggtgccgtaaagcactaaatcggaaccctaaagggagcccccgatttagagcttgacggggaaagccggcgaacgtggcgagaaaggaagggaagaaagcgaaaggagcgggcgctagggcgctggcaagtgtagcggtcacgctgcgcgtaaccaccacacccgccgcgcttaatgcgccgctacagggcgcgtactatggttgctttgacgtatgcggtgtgaaataccgcacagatgcgtaaggagaaaataccgcatcaggcgtcaggtggcacttttcggggaaatgtgcgcggaacccctatttgtttatttttctaaatacattcaaatatgtatccgctcatgagacaataaccctgataaatgcttcaataatattgaaaaaggaagagtatgagtattcaacatttccgtgtcgcccttattcccttttttgcggcattttgccttcctgtttttgctcacccagaaacgctggtgaaagtaaaagatgctgaagatcagttgggtgcacgagtgggttacatcgaactggatctcaacagcggtaagatccttgagagttttcgccccgaagaacgttttccaatgatgagcacttttaaagttctgctatgtggcgcggtattatcccgtattgacgccgggcaagagcaactcggtcgccgcatacactattctcagaatgacttggttgagtactcaccagtcacagaaaagcatcttacggatggcatgacagtaagagaattatgcagtgctgccataaccatgagtgataacactgcggccaacttacttctgacaacgatcggaggaccgaaggagctaaccgcttttttgcacaacatgggggatcatgtaactcgccttgatcgttgggaaccggagctgaatgaagccataccaaacgacgagcgtgacaccacgatgcctgtagcaatggcaacaacgttgcgcaaactattaactggcgaactacttactctagcttcccggcaacaattaatagactggatggaggcggataaagttgcaggaccacttctgcgctcggcccttccggctggctggtttattgctgataaatctggagccggtgagcgtgggtctcgcggtatcattgcagcactggggccagatggtaagccctcccgtatcgtagttatctacacgacggggagtcaggcaactatggatgaacgaaatagacagatcgctgagataggtgcctcactgattaagcattggtaactgtcagaccaagtttactcatatatactttagattgatttaaaacttcatttttaatttaaaaggatctaggtgaagatcctttttgataatctcatgaccaaaatcccttaacgtgagttttcgttccactgagcgtcagaccccgtagaaaagatcaaaggatcttcttgagatcctttttttctgcgcgtaatctgctgcttgcaaacaaaaaaaccaccgctaccagcggtggtttgtttgccggatcaagagctaccaactctttttccgaaggtaactggcttcagcagagcgcagataccaaatactgttcttctagtgtagccgtagttaggccaccacttcaagaactctgtagcaccgcctacatacctcgctctgctaatcctgttaccagtggctgctgccagtggcgataagtcgtgtcttaccgggttggactcaagacgatagttaccggataaggcgcagcggtcgggctgaacggggggttcgtgcacacagcccagcttggagcgaacgacctacaccgaactgagatacctacagcgtgagctatgagaaagcgccacgcttcccgaagggagaaaggcggacaggtatccggtaagcggcagggtcggaacaggagagcgcacgagggagcttccagggggaaacgcctggtatctttatagtcctgtcgggtttcgccacctctgacttgagcgtcgatttttgtgatgctcgtcaggggggcggagcctatggaaaaacgccagcaacgcggcctttttacggttcctggccttttgctggccttttgctcacatagtcatgccccgcgcccaccggaaggagctgactgggttgaaggctctcaagggcatcggtcgagatcccggtgcctaatgagtgagctaacttacattaattgcgttgcgctcactgcccgctttccagtcgggaaacctgtcgtgccagctgcattaatgaatcggccaacgcgcggggagaggcggtttgcgtattgggcgccagggtggtttttcttttcaccagtgagacgggcaacagctgattgcccttcaccgcctggccctgagagagttgcagcaagcggtccacgctggtttgccccagcaggcgaaaatcctgtttgatggtggttaacggcgggatataacatgagctgtcttcggtatcgtcgtatcccactaccgagatatccgcaccaacgcgcagcccggactcggtaatggcgcgcattgcgcccagcgccatctgatcgttggcaaccagcatcgcagtgggaacgatgccctcattcagcatttgcatggtttgttgaaaaccggacatggcactccagtcgccttcccgttccgctatcggctgaatttgattgcgagtgagatatttatgccagccagccagacgcagacgcgccgagacagaacttaatgggcccgctaacagcgcgatttgctggtgacccaatgcgaccagatgctccacgcccagtcgcgtaccgtcttcatgggagaaaataatactgttgatgggtgtctggtcagagacatcaagaaataacgccggaacattagtgcaggcagcttccacagcaatggcatcctggtcatccagcggatagttaatgatcagcccactgacgcgttgcgcgagaagattgtgcaccgccgctttacaggcttcgacgccgcttcgttctaccatcgacaccaccacgctggcacccagttgatcggcgcgagatttaatcgccgcgacaatttgcgacggcgcgtgcagggccagactggaggtggcaacgccaatcagcaacgactgtttgcccgccagttgttgtgccacgcggttgggaatgtaattcagctccgccatcgccgcttccactttttcccgcgttttcgcagaaacgtggctggcctggttcaccacgcgggaaacggtctgataagagacaccggcatactctgcgacatcgtataacgttactggtttcacattcaccaccctgaattgactctcttccgggcgctatcatgccataccgcgaaaggttttgcgccattcgatggtgtccgggatctcgacgctctcccttatgcgactcctgcattaggaagcagcccagtagtaggttgaggccgttgagcaccgccgccgc

SEQ ID NO: 5 - DNA, 5375 bp, Artificial Sequence
  Recombinant vector containing a rCod UNG hydrolase
aaggaatggtgtggccgattaatcataaatatgaaaaataattgttgcatcacccgccaatgcgtggcttaatgcacatcaaattgtgagcggataacaatttgatgtgctagcgcatatccagtgtagtaaggcaagtcccttcaagagttatcgttgatacccctcgtagtgcacattcctttaacgcttcaaaatctgtaaagcacgccatatcgccgaaaggcacacttaattattaagaggtaatacaccatgaatcacaaagtgcatcatcatcatcatcatatcgaaggtaggcatatgggcggtggcggtagcggcggtggcggtagcggtatgtcggactcagaagtcaatcaagaagctaagccagaggtcaagccagaagtcaagcctgagactcacatcaatttaaaggtgtccgatggatcttcagagatcttcttcaagatcaaaaagaccactcctttaagaaggctgatggaagcgttcgctaaaagacagggtaaggaaatggactccttaagattcttgtacgacggtattagaattcaagctgatcagacccctgaagatttggacatggaggataacgatattattgaggctcacagagaacagattggtggtactagtgagctcggtaccatgttcggagagacttggagaagagagctggctgcagagtttgaaaagccatacttcaaacaattgatgtcctttgtagctgatgagaggagccgtcacaccgtctacccaccggctgatcaagtgtacagttggacagagatgtgtgacattcaagatgtgaaagtagtgattctaggccaggacccttaccacggtcccaaccaagcacatggactctgtttcagtgtgcaaaagccagttccccctccccccagtctcgtgaacatatacaaagaattgtgtaccgacattgatggcttcaagcatcctggacatggagatctaagcggatgggcaaaacaaggggtgctgctgcttaacgcggtgctgaccgtgcgggcccatcaggccaactcccacaaggacagaggctgggagaccttcaccgacgctgtgatcaagtggctgagcgtcaaccgggaaggagtggttttcctgttgtggggctcatacgcccataagaagggagcgaccatcgacaggaaacgtcaccatgtcttgcaagctgttcatccatctcctttgtctgctcatcgtgggttccttggttgtaagcacttctccaaggctaacgggctgctgaaactatctgggacggagcctataaactggagagcactctaatgcagtctagataggtaatctctgcttaaaagcacagaatctaagatccctgccatttggcggggatttttttatttgttttcaggaaataaataatcgatcgcgtaataaaatctattattatttttgtgaagaataaatttgggtgcaatgagaatgcgcaggccctttcgtctcgcgcgtttcggtgatgacggtgaaaacctctgacacatgcagctcccggagacggtcacagcttgtctgtaagcggatgccgggagcagacaagcccgtcagggcgcgtcagcgggtgttggcgggtgtcggggctggcttaactatgcggcatcagagcagattgtactgagagtgcaccataaaattgtaaacgttaatattttgttaaaattcgcgttaaatttttgttaaatcagctcattttttaaccaataggccgaaatcggcaaaatcccttataaatcaaaagaatagcccgagatagggttgagtgttgttccagtttggaacaagagtccactattaaagaacgtggactccaacgtcaaagggcgaaaaaccgtctatcagggcgatggcccactacgtgaaccatcacccaaatcaagttttttggggtcgaggtgccgtaaagcactaaatcggaaccctaaagggagcccccgatttagagcttgacggggaaagccggcgaacgtggcgagaaaggaagggaagaaagcgaaaggagcgggcgctagggcgctggcaagtgtagcggtcacgctgcgcgtaaccaccacacccgccgcgcttaatgcgccgctacagggcgcgtactatggttgctttgacgtatgcggtgtgaaataccgcacagatgcgtaaggagaaaataccgcatcaggcgtcaggtggcacttttcggggaaatgtgcgcggaacccctatttgtttatttttctaaatacattcaaatatgtatccgctcatgagacaataaccctgataaatgcttcaataatattgaaaaaggaagagtatgagtattcaacatttccgtgtcgcccttattcccttttttgcggcattttgccttcctgtttttgctcacccagaaacgctggtgaaagtaaaagatgctgaagatcagttgggtgcacgagtgggttacatcgaactggatctcaacagcggtaagatccttgagagttttcgccccgaagaacgttttccaatgatgagcacttttaaagttctgctatgtggcgcggtattatcccgtattgacgccgggcaagagcaactcggtcgccgcatacactattctcagaatgacttggttgagtactcaccagtcacagaaaagcatcttacggatggcatgacagtaagagaattatgcagtgctgccataaccatgagtgataacactgcggccaacttacttctgacaacgatcggaggaccgaaggagctaaccgcttttttgcacaacatgggggatcatgtaactcgccttgatcgttgggaaccggagctgaatgaagccataccaaacgacgagcgtgacaccacgatgcctgtagcaatggcaacaacgttgcgcaaactattaactggcgaactacttactctagcttcccggcaacaattaatagactggatggaggcggataaagttgcaggaccacttctgcgctcggcccttccggctggctggtttattgctgataaatctggagccggtgagcgtgggtctcgcggtatcattgcagcactggggccagatggtaagccctcccgtatcgtagttatctacacgacggggagtcaggcaactatggatgaacgaaatagacagatcgctgagataggtgcctcactgattaagcattggtaactgtcagaccaagtttactcatatatactttagattgatttaaaacttcatttttaatttaaaaggatctaggtgaagatcctttttgataatctcatgaccaaaatcccttaacgtgagttttcgttccactgagcgtcagaccccgtagaaaagatcaaaggatcttcttgagatcctttttttctgcgcgtaatctgctgcttgcaaacaaaaaaaccaccgctaccagcggtggtttgtttgccggatcaagagctaccaactctttttccgaaggtaactggcttcagcagagcgcagataccaaatactgttcttctagtgtagccgtagttaggccaccacttcaagaactctgtagcaccgcctacatacctcgctctgctaatcctgttaccagtggctgctgccagtggcgataagtcgtgtcttaccgggttggactcaagacgatagttaccggataaggcgcagcggtcgggctgaacggggggttcgtgcacacagcccagcttggagcgaacgacctacaccgaactgagatacctacagcgtgagctatgagaaagcgccacgcttcccgaagggagaaaggcggacaggtatccggtaagcggcagggtcggaacaggagagcgcacgagggagcttccagggggaaacgcctggtatctttatagtcctgtcgggtttcgccacctctgacttgagcgtcgatttttgtgatgctcgtcaggggggcggagcctatggaaaaacgccagcaacgcggcctttttacggttcctggccttttgctggccttttgctcacatagtcatgccccgcgcccaccggaaggagctgactgggttgaaggctctcaagggcatcggtcgagatcccggtgcctaatgagtgagctaacttacattaattgcgttgcgctcactgcccgctttccagtcgggaaacctgtcgtgccagctgcattaatgaatcggccaacgcgcggggagaggcggtttgcgtattgggcgccagggtggtttttcttttcaccagtgagacgggcaacagctgattgcccttcaccgcctggccctgagagagttgcagcaagcggtccacgctggtttgccccagcaggcgaaaatcctgtttgatggtggttaacggcgggatataacatgagctgtcttcggtatcgtcgtatcccactaccgagatatccgcaccaacgcgcagcccggactcggtaatggcgcgcattgcgcccagcgccatctgatcgttggcaaccagcatcgcagtgggaacgatgccctcattcagcatttgcatggtttgttgaaaaccggacatggcactccagtcgccttcccgttccgctatcggctgaatttgattgcgagtgagatatttatgccagccagccagacgcagacgcgccgagacagaacttaatgggcccgctaacagcgcgatttgctggtgacccaatgcgaccagatgctccacgcccagtcgcgtaccgtcttcatgggagaaaataatactgttgatgggtgtctggtcagagacatcaagaaataacgccggaacattagtgcaggcagcttccacagcaatggcatcctggtcatccagcggatagttaatgatcagcccactgacgcgttgcgcgagaagattgtgcaccgccgctttacaggcttcgacgccgcttcgttctaccatcgacaccaccacgctggcacccagttgatcggcgcgagatttaatcgccgcgacaatttgcgacggcgcgtgcagggccagactggaggtggcaacgccaatcagcaacgactgtttgcccgccagttgttgtgccacgcggttgggaatgtaattcagctccgccatcgccgcttccactttttcccgcgttttcgcagaaacgtggctggcctggttcaccacgcgggaaacggtctgataagagacaccggcatactctgcgacatcgtataacgttactggtttcacattcaccaccctgaattgactctcttccgggcgctatcatgccataccgcgaaaggttttgcgccattcgatggtgtccgggatctcgacgctctcccttatgcgactcctgcattaggaagcagcccagtagtaggttgaggccgttgagcaccgccgccgc